European Patent Application EP 4 299 729 A1, published January 3, 2024. Title: Oncolytic Virus and Uses Thereof. Applicant: SillaJen, Inc. The sequence listing filed with the application follows.

SEQUENCE LISTING (38 sequences)

SEQ ID NO: 1 - DNA, 1055 bp, Artificial Sequence
  human CD55
tgaccgtcgcgcggccgagcgtgcccgcggcgctgcccctcctcggggagctgccccggctgctgctgctggtgctgttgtgcctgccggccgtgtggggtgactgtggccttcccccagatgtacctaatgcccagccagctttggaaggccgtacaagttttcccgaggatactgtaataacgtacaaatgtgaagaaagctttgtgaaaattcctggcgagaaggactcagtgatctgccttaagggcagtcaatggtcagatattgaagagttctgcaatcgtagctgcgaggtgccaacaaggctaaattctgcatccctcaaacagccttatatcactcagaattattttccagtcggtactgttgtggaatatgagtgccgtccaggttacagaagagaaccttctctatcaccaaaactaacttgccttcagaatttaaaatggtccacagcagtcgaattttgtaaaaagaaatcatgccctaatccgggagaaatacgaaatggtcagattgatgtaccaggtggcatattatttggtgcaaccatctccttctcatgtaacacagggtacaaattatttggctcgacttctagtttttgtcttatttcaggcagctctgtccagtggagtgacccgttgccagagtgcagagaaatttattgtccagcaccaccacaaattgacaatggaataattcaaggggaacgtgaccattatggatatagacagtctgtaacgtatgcatgtaataaaggattcaccatgattggagagcactctatttattgtactgtgaataatgatgaaggagagtggagtggcccaccacctgaatgcagaggaaaatctctaacttccaaggtcccaccaacagttcagaaacctaccacagtaaatgttccaactacagaagtctcaccaacttctcagaaaaccaccacaaaaaccaccacaccaaatgctcaagcaacacggagtacacctgtttccaggacaaccaagcattttcatgaaacaaccccaaataaaggaagtggaaccact

SEQ ID NO: 2 - protein, 352 aa, Artificial Sequence
  human CD55
MTVARPSVPAALPLLGELPRLLLLVLLCLPAVWGDCGLPPDVPNAQPALEGRTSFPEDTVITYKCEESFVKIPGEKDSVICLKGSQWSDIEEFCNRSCEVPTRLNSASLKQPYITQNYFPVGTVVEYECRPGYRREPSLSPKLTCLQNLKWSTAVEFCKKKSCPNPGEIRNGQIDVPGGILFGATISFSCNTGYKLFGSTSSFCLISGSSVQWSDPLPECREIYCPAPPQIDNGIIQGERDHYGYRQSVTYACNKGFTMIGEHSIYCTVNNDEGEWSGPPPECRGKSLTSKVPPTVQKPTTVNVPTTEVSPTSQKTTTKTTTPNAQATRSTPVSRTTKHFHETTPNKGSGTT

SEQ ID NO: 3 - DNA, 40 bp, Artificial Sequence
  pSEL
aaaaattgaaattttattttttttttttggaatataaata

SEQ ID NO: 4 - DNA, 32 bp, Artificial Sequence
  pLate
ttttttttttttttttttttggcatataaata

SEQ ID NO: 5 - protein, 29 aa, Artificial Sequence
  D8L transmembrane domain
FAIIAIVFVFILTAILFFMSRRYSREKQN

SEQ ID NO: 6 - DNA, 87 bp, Artificial Sequence
  D8L transmembrane domain
ttcgcaattattgccatagtattcgtgtttatacttaccgctattctcttttttatgagtcgacgatattcgcgagaaaaacaaaac

SEQ ID NO: 7 - protein, 35 aa, Artificial Sequence
  A16L transmembrane domain
LGAAITLVVISVIFYFISIYSRPKIKTNDINVRRR

SEQ ID NO: 8 - DNA, 105 bp, Artificial Sequence
  A16L transmembrane domain
ttgggcgcggccataacattggttgtaatatctgttattttctattttatatctatttattcgcgtactaaaattaaaacaaatgatataaatgttcgtagacga

SEQ ID NO: 9 - protein, 37 aa, Artificial Sequence
  F9L transmembrane domain
PWFLVGVAIILVIFTVAICSIRRNLALKYRYGTFLYV

SEQ ID NO: 10 - DNA, 111 bp, Artificial Sequence
  F9L transmembrane domain
ccgtggtttctagtgggtgtagcaattattctagttatttttactgtagctatttgttctattagacgaaatctggctcttaaatacagatacggaacgtttttatacgtt

SEQ ID NO: 11 - protein, 21 aa, Artificial Sequence
  G9R transmembrane domain
LKLHLISLLSLLVIWILIVAI

SEQ ID NO: 12 - DNA, 63 bp, Artificial Sequence
  G9R transmembrane domain
ctaaaattgcatttgatcagtttattatctctcttggtaatatggatactaattgtagctatt

SEQ ID NO: 13 - protein, 40 aa, Artificial Sequence
  H3L transmembrane domain
LFDINVIGLIVILFIMFMLIFNVKSKLLWFLTGTFVTAFI

SEQ ID NO: 14 - DNA, 120 bp, Artificial Sequence
  H3L transmembrane domain
ttgtttgatattaatgttataggtttgattgtaattttgtttattatgtttatgctcatctttaacgttaaatctaagctgttatggttccttacaggaacattcgttaccgcatttatc

SEQ ID NO: 15 - protein, 67 aa, Artificial Sequence
  L1R transmembrane domain
VQFYMIVIGVIILAALFMYYAKRMLFTSTNDKIKLILANKENVHWTTYMDTFFRTSPMVIATTDMQN

SEQ ID NO: 16 - DNA, 201 bp, Artificial Sequence
  L1R transmembrane domain
gttcagttttatatgattgttatcggtgttataatattggcagcgttgtttatgtactatgccaagcgtatgttgttcacatccaccaatgataaaatcaaacttattttagccaataaggaaaacgtccattggactacttacatggacacattctttagaacttctccgatggttattgctaccacggatatgcaaaac

SEQ ID NO: 17 - protein, 21 aa, Artificial Sequence
  A9L transmembrane domain
FVVVRAIASMIMYLVLGIALL

SEQ ID NO: 18 - DNA, 63 bp, Artificial Sequence
  A9L transmembrane domain
ttcgtcgttgttagagccattgcgagcatgataatgtatttagtattaggtatagcattgctg

SEQ ID NO: 19 - protein, 21 aa, Artificial Sequence
  A13L transmembrane domain
MIGILLLIGICVAVTVAILYA

SEQ ID NO: 20 - DNA, 63 bp, Artificial Sequence
  A13L transmembrane domain
atgattggtattcttttgttgatcggtatttgcgtagcagttaccgtcgccatcctatatgcg

SEQ ID NO: 21 - protein, 21 aa, Artificial Sequence
  A21L transmembrane domain
MITLFLILCYFILIFNIIVPA

SEQ ID NO: 22 - DNA, 63 bp, Artificial Sequence
  A21L transmembrane domain
atgataactttatttttaatcctatgttatttcattcttatttttaatattatagtacctgca

SEQ ID NO: 23 - protein, 21 aa, Artificial Sequence
  A28L transmembrane domain
MNSLSIFFIVVATAAVCLLFI

SEQ ID NO: 24 - DNA, 63 bp, Artificial Sequence
  A28L transmembrane domain
atgaactctctatcaattttttttattgtggtagcgacggctgcggtgtgtttactttttatc

SEQ ID NO: 25 - protein, 17 aa, Artificial Sequence
  E10R transmembrane domain
AVWTIIFIVLSQAGLDG

SEQ ID NO: 26 - DNA, 51 bp, Artificial Sequence
  E10R transmembrane domain
gccgtatggaccattatttttatagtactttcgcaagcgggtttagacggc

SEQ ID NO: 27 - protein, 21 aa, Artificial Sequence
  G3L transmembrane domain
MASLLYLILFLLFVCISYYFT

SEQ ID NO: 28 - DNA, 63 bp, Artificial Sequence
  G3L transmembrane domain
atggcatctttattatatcttattttatttttgttattcgtatgtatttcttattattttaca

SEQ ID NO: 29 - protein, 21 aa, Artificial Sequence
  H2R transmembrane domain
TSTLIFFVIILAISALLLWFQ

SEQ ID NO: 30 - DNA, 63 bp, Artificial Sequence
  H2R transmembrane domain
acatcaacacttatattctttgttattatattggcaattagtgcgctattactctggtttcag

SEQ ID NO: 31 - protein, 21 aa, Artificial Sequence
  I2L transmembrane domain
YWLIIIFFIVLILLLLIYLYL

SEQ ID NO: 32 - DNA, 63 bp, Artificial Sequence
  I2L transmembrane domain
tattggttaattattattttttttatagttcttattctactactattgatatatttgtattta

SEQ ID NO: 33 - protein, 21 aa, Artificial Sequence
  J5L transmembrane domain
IIDIKWLPIGLLALAILILAF

SEQ ID NO: 34 - DNA, 63 bp, Artificial Sequence
  J5L transmembrane domain
attatagatatcaaatggcttccgattggattactagcgttagctattttaatattagcattt

SEQ ID NO: 35 - protein, 21 aa, Artificial Sequence
  L5R transmembrane domain
IVLFEVFVVFILIYVFFRSEL

SEQ ID NO: 36 - DNA, 63 bp, Artificial Sequence
  L5R transmembrane domain
atagttttatttgaagtattcgttgtattcattctaatatatgtattttttagatctgaatta

SEQ ID NO: 37 - protein, 21 aa, Artificial Sequence
  O3L transmembrane domain
LVVIMFFIAFAFCSWLSYSYL

SEQ ID NO: 38 - DNA, 63 bp, Artificial Sequence
  O3L transmembrane domain
ctcgtcgtaattatgttttttatagcgtttgccttctgtagttggctatcatatagctatctg